European Patent Application EP 4 180 447 A1, published May 17, 2023. Title: Carrier Protein Subjected to Site-directed Mutation and Use Thereof in Preparation of Vaccine. Applicant: Cansino Biologics Inc. The sequence listing filed with the application follows.

SEQUENCE LISTING (57 sequences)

SEQ ID NO: 1 - protein, 261 aa, Unknown
  Amino acid sequence of MenB V.155
CGSSGGGGSGGGGVTADIGTGLADALTAPLDHKDKGLKSLTLEDSISQNGTLTLSAQGAEKTYGNGDSLNTGKLKNDKVSRFDFIRQIEVDGQLITLESGEFQVYKQSHSALTALQTEQEQDPEHSEKMVAKRRFRIGDIAGEHTSFDKLPKDVMATYRGTAFGSDDAGGKLTYTIDFAAKQGHGKIEHLKSPELNVDLAVAYIKPDEKHHAVISGSVLYNQDEKGSYSLGIFGEKAQEVAGSAEVETANGIHHIGLAAKQ

SEQ ID NO: 2 - protein, 255 aa, Unknown
  Amino acid sequence of MenB V2.16
CGSSGGGGVAADIGAGLADALTAPLDHKDKSLQSLTLDQSVRKNEKLKLAAQGAEKTYGNGDSLNTGKLKNDKVSRFDFIRQIEVDGQLITLESGEFQIYKQDHSAVVALQIEKINNPDKIDSLINQRSFLVSGLGGEHTAFNQLPDGKAEYHGKAFSSDDAGGKLTYTIDFAAKQGHGKIEHLKTPEQNVELAAAELKADEKSHAVILGDTRYGSEEKGTYHLALFGDRAQEIAGSATVKIGEKVHEIGIAGKQ

SEQ ID NO: 3 - protein, 258 aa, Unknown
  Amino acid sequence of MenB V3.45
CGSSGGGGVAADIGTGLADALTAPLDHKDKGLKSLTLEDSISQNGTLTLSAQGAEKTFKVGDKDNSLNTGKLKNDKISRFDFVQKIEVDGQTITLASGEFQIYKQDHSAVVALQIEKINNPDKIDSLINQRSFLVSGLGGEHTAFNQLPSGKAEYHGKAFSSDDAGGKLTYTIDFAAKQGHGKIEHLKTPEQNVELASAELKADEKSHAVILGDTRYGSEEKGTYHLALFGDRAQEIAGSATVKIREKVHEIGIAGKQ

SEQ ID NO: 4 - DNA, 43 bp, Artificial Sequence
  Forward primer for MenB V1.55 G2 mutation site
ggagatataccatgggttgttagagcagcggtggtggtggtag

SEQ ID NO: 5 - DNA, 23 bp, Artificial Sequence
  Reverse primer for MenB V1.55 G2 mutation site
ctaacaacccatggtatatctcc

SEQ ID NO: 6 - DNA, 43 bp, Artificial Sequence
  Forward primer for MenB V1.55 S3 mutation site
gatataccatgggttgtggttagagcggtggtggtggtagtgg

SEQ ID NO: 7 - DNA, 23 bp, Artificial Sequence
  Reverse primer for MenB V1.55 S3 mutation site
ctaaccacaacccatggtatatc

SEQ ID NO: 8 - DNA, 43 bp, Artificial Sequence
  Forward primer for MenB V1.55 S4 mutation site
ataccatgggttgtggtagctagggtggtggtggtagtggtgg

SEQ ID NO: 9 - DNA, 23 bp, Artificial Sequence
  Reverse primer for MenB V1.55 S4 mutation site
ctagctaccacaacccatggtat

SEQ ID NO: 10 - DNA, 43 bp, Artificial Sequence
  Forward primer for MenB V1.55 G5 mutation site
ccatgggttgtggtagcagctagggtggtggtagtggtggcgg

SEQ ID NO: 11 - DNA, 23 bp, Artificial Sequence
  Reverse primer for MenB V1.55 G5 mutation site
ctagctgctaccacaacccatgg

SEQ ID NO: 12 - DNA, 43 bp, Artificial Sequence
  Forward primer for MenB V1.55 G6 mutation site
tgggttgtggtagcagcggttagggtggtagtggtggcggtgg

SEQ ID NO: 13 - DNA, 23 bp, Artificial Sequence
  Reverse primer for MenB V1.55 G6 mutation site
ctaaccgctgctaccacaaccca

SEQ ID NO: 14 - DNA, 43 bp, Artificial Sequence
  Forward primer for MenB V1.55 G7 mutation site
gttgtggtagcagcggtggttagggtagtggtggcggtggtgt

SEQ ID NO: 15 - DNA, 23 bp, Artificial Sequence
  Reverse primer for MenB V1.55 G7 mutation site
ctaaccaccgctgctaccacaac

SEQ ID NO: 16 - DNA, 43 bp, Artificial Sequence
  Forward primer for MenB V1.55 G8 mutation site
gtggtagcagcggtggtggttagagtggtggcggtggtgttac

SEQ ID NO: 17 - DNA, 23 bp, Artificial Sequence
  Reverse primer for MenB V1.55 G8 mutation site
ctaaccaccaccgctgctaccac

SEQ ID NO: 18 - DNA, 43 bp, Artificial Sequence
  Forward primer for MenB V1.55 S9 mutation site
gtagcagcggtggtggtggttagggtggcggtggtgttaccgc

SEQ ID NO: 19 - DNA, 23 bp, Artificial Sequence
  Reverse primer for MenB V1.55 S9 mutation site
ctaaccaccaccaccgctgctac

SEQ ID NO: 20 - DNA, 43 bp, Artificial Sequence
  Forward primer for MenB V1.55 G10 mutation site
gcagcggtggtggtggtagttagggcggtggtgttaccgcaga

SEQ ID NO: 21 - DNA, 23 bp, Artificial Sequence
  Reverse primer for MenB V1.55 G10 mutation site
ctaactaccaccaccaccgctgc

SEQ ID NO: 22 - DNA, 43 bp, Artificial Sequence
  Forward primer for MenB V2.16 G2 mutation site
ggagatataccatgggttgttagagcagcggtggtggtggcgt

SEQ ID NO: 23 - DNA, 23 bp, Artificial Sequence
  Reverse primer for MenB V2.16 G2 mutation site
ctaacaacccatggtatatctcc

SEQ ID NO: 24 - DNA, 43 bp, Artificial Sequence
  Forward primer for MenB V2.16 S3 mutation site
gatataccatgggttgtggttagagcggtggtggtggcgttgc

SEQ ID NO: 25 - DNA, 23 bp, Artificial Sequence
  Reverse primer for MenB V2.16 S3 mutation site
ctaaccacaacccatggtatatc

SEQ ID NO: 26 - DNA, 43 bp, Artificial Sequence
  Forward primer for MenB V2.16 S4 mutation site
ataccatgggttgtggtagctagggtggtggtggcgttgcagc

SEQ ID NO: 27 - DNA, 23 bp, Artificial Sequence
  Reverse primer for MenB V2.16 S4 mutation site
ctagctaccacaacccatggtat

SEQ ID NO: 28 - DNA, 43 bp, Artificial Sequence
  Forward primer for MenB V2.16 G5 mutation site
ccatgggttgtggtagcagctagggtggtggcgttgcagcaga

SEQ ID NO: 29 - DNA, 23 bp, Artificial Sequence
  Reverse primer for MenB V2.16 G5 mutation site
ctagctgctaccacaacccatgg

SEQ ID NO: 30 - DNA, 43 bp, Artificial Sequence
  Forward primer for MenB V2.16 G6 mutation site
tgggttgtggtagcagcggttagggtggcgttgcagcagatat

SEQ ID NO: 31 - DNA, 23 bp, Artificial Sequence
  Reverse primer for MenB V2.16 G6 mutation site
ctaaccgctgctaccacaaccca

SEQ ID NO: 32 - DNA, 43 bp, Artificial Sequence
  Forward primer for MenB V2.16 G7 mutation site
gttgtggtagcagcggtggttagggcgttgcagcagatattgg

SEQ ID NO: 33 - DNA, 23 bp, Artificial Sequence
  Reverse primer for MenB V2.16 G7 mutation site
ctaaccaccgctgctaccacaac

SEQ ID NO: 34 - DNA, 43 bp, Artificial Sequence
  Forward primer for MenB V2.16 G8 mutation site
gtggtagcagcggtggtggttaggttgcagcagatattggtgc

SEQ ID NO: 35 - DNA, 23 bp, Artificial Sequence
  Reverse primer for MenB V2.16 G8 mutation site
ctaaccaccaccgctgctaccac

SEQ ID NO: 36 - DNA, 43 bp, Artificial Sequence
  Forward primer for MenB V2.16 V9 mutation site
gtagcagcggtggtggtggctaggcagcagatattggtgcagg

SEQ ID NO: 37 - DNA, 23 bp, Artificial Sequence
  Reverse primer for MenB V2.16 V9 mutation site
ctagccaccaccaccgctgctac

SEQ ID NO: 38 - DNA, 43 bp, Artificial Sequence
  Forward primer for MenB V2.16 A10 mutation site
gcagcggtggtggtggcgtttaggcagatattggtgcaggtct

SEQ ID NO: 39 - DNA, 23 bp, Artificial Sequence
  Reverse primer for MenB V2.16 A10 mutation site
ctaaacgccaccaccaccgctgc

SEQ ID NO: 40 - DNA, 43 bp, Artificial Sequence; identical to SEQ ID NO: 22
  Forward primer for MenB V3.45 G2 mutation site

SEQ ID NO: 41 - DNA, 23 bp, Artificial Sequence
  Reverse primer for MenB V3.45 G2 mutation site
ctaacaacccatggtatatctcc

SEQ ID NO: 42 - DNA, 43 bp, Artificial Sequence; identical to SEQ ID NO: 24
  Forward primer for MenB V3.45 S3 mutation site

SEQ ID NO: 43 - DNA, 23 bp, Artificial Sequence
  Reverse primer for MenB V3.45 S3 mutation site
ctaaccacaacccatggtatatc

SEQ ID NO: 44 - DNA, 43 bp, Artificial Sequence; identical to SEQ ID NO: 26
  Forward primer for MenB V3.45 S4 mutation site

SEQ ID NO: 45 - DNA, 23 bp, Artificial Sequence
  Reverse primer for MenB V3.45 S4 mutation site
ctagctaccacaacccatggtat

SEQ ID NO: 46 - DNA, 43 bp, Artificial Sequence; identical to SEQ ID NO: 28
  Forward primer for MenB V3.45 G5 mutation site

SEQ ID NO: 47 - DNA, 23 bp, Artificial Sequence
  Reverse primer for MenB V3.45 G5 mutation site
ctagctgctaccacaacccatgg

SEQ ID NO: 48 - DNA, 43 bp, Artificial Sequence; identical to SEQ ID NO: 30
  Forward primer for MenB V3.45 G6 mutation site

SEQ ID NO: 49 - DNA, 23 bp, Artificial Sequence
  Reverse primer for MenB V3.45 G6 mutation site
ctaaccgctgctaccacaaccca

SEQ ID NO: 50 - DNA, 43 bp, Artificial Sequence; identical to SEQ ID NO: 32
  Forward primer for MenB V3.45 G7 mutation site

SEQ ID NO: 51 - DNA, 23 bp, Artificial Sequence
  Reverse primer for MenB V3.45 G7 mutation site
ctaaccaccgctgctaccacaac

SEQ ID NO: 52 - DNA, 43 bp, Artificial Sequence
  Forward primer for MenB V3.45 G8 mutation site
gtggtagcagcggtggtggttaggttgcagcagatattggcac

SEQ ID NO: 53 - DNA, 23 bp, Artificial Sequence
  Reverse primer for MenB V3.45 G8 mutation site
ctaaccaccaccgctgctaccac

SEQ ID NO: 54 - DNA, 43 bp, Artificial Sequence
  Forward primer for MenB V3.45 V9 mutation site
gtagcagcggtggtggtggctaggcagcagatattggcaccgg

SEQ ID NO: 55 - DNA, 23 bp, Artificial Sequence
  Reverse primer for MenB V3.45 V9 mutation site
ctagccaccaccaccgctgctac

SEQ ID NO: 56 - DNA, 43 bp, Artificial Sequence
  Forward primer for MenB V3.45 A10 mutation site
gcagcggtggtggtggcgtttaggcagatattggcaccggtct

SEQ ID NO: 57 - DNA, 23 bp, Artificial Sequence
  Reverse primer for MenB V3.45 A10 mutation site
ctaaacgccaccaccaccgctgc